European Patent Application EP 4 620 482 A1, published September 24, 2025. Title: FLAGELLIN-RELATED PEPTIDES AND USES THEREOF. Applicant: ISTITUTO EUROPEO DI ONCOLOGIA S.R.L. The sequence listing filed with the application follows.

SEQUENCE LISTING (143 sequences)

SEQ ID NO: 1 - protein, 9 aa, Roseburia sp.
KMSYEDIEL

SEQ ID NO: 2 - protein, 9 aa, Roseburia sp.
MPKDGAAFI

SEQ ID NO: 3 - protein, 9 aa, Roseburia sp.
ALNETSAIL

SEQ ID NO: 4 - protein, 9 aa, Roseburia sp.
ILAQAGQSM

SEQ ID NO: 5 - protein, 9 aa, Clostridium sp.
ILAQAGTSM

SEQ ID NO: 6 - protein, 9 aa, Roseburia sp.
NEFNADLLM

SEQ ID NO: 7 - protein, 9 aa, Clostridium sp.
TEFNGQKLL

SEQ ID NO: 8 - protein, 9 aa, Clostridium sp.
SVRGRLGAF

SEQ ID NO: 9 - protein, 9 aa, Clostridium sp.
FPELKHFTM

SEQ ID NO: 10 - protein, 9 aa, Roseburia sp.
GLDALNNLL

SEQ ID NO: 11 - protein, 9 aa, unidentified
STEKLSSGY

SEQ ID NO: 12 - protein, 9 aa, unidentified
RMLNVTTSA

SEQ ID NO: 13 - protein, 9 aa, unidentified
ALTEVHSML

SEQ ID NO: 14 - protein, 9 aa, unidentified
SMLQRMNEL

SEQ ID NO: 15 - protein, 9 aa, unidentified
EVHSMLQRM

SEQ ID NO: 16 - protein, 9 aa, Roseburia sp.
VLTTVRVPK

SEQ ID NO: 17 - protein, 9 aa, Roseburia sp.
IIINMSNNK

SEQ ID NO: 18 - protein, 9 aa, Roseburia sp.
MKQEDTFVL

SEQ ID NO: 19 - protein, 9 aa, Roseburia sp.
SHIMWLQSM

SEQ ID NO: 20 - protein, 9 aa, Roseburia sp.
FPDMQKFTL

SEQ ID NO: 21 - protein, 9 aa, Roseburia sp.
KGSKSHIMW

SEQ ID NO: 22 - protein, 9 aa, Roseburia sp.
TLMPCCPAV

SEQ ID NO: 23 - protein, 9 aa, Roseburia sp.
YLNPVIEKA

SEQ ID NO: 24 - protein, 9 aa, Roseburia sp.
YLENSFEEL

SEQ ID NO: 25 - protein, 9 aa, Roseburia sp.
WLLDGQKEI

SEQ ID NO: 26 - protein, 9 aa, Roseburia sp.
QAYNPLMRK

SEQ ID NO: 27 - protein, 9 aa, Roseburia sp.
VFPREVHRF

SEQ ID NO: 28 - protein, 9 aa, Roseburia sp.
EMADRMHEF

SEQ ID NO: 29 - protein, 9 aa, Roseburia sp.
LPQKKNLSA

SEQ ID NO: 30 - protein, 9 aa, Roseburia sp.
YIREKLTEL

SEQ ID NO: 31 - protein, 9 aa, Roseburia sp.
NPLMRKFLI

SEQ ID NO: 32 - protein, 9 aa, Roseburia sp.
RMHEFESEF

SEQ ID NO: 33 - protein, 9 aa, Roseburia sp.
VLSETCAVF

SEQ ID NO: 34 - protein, 9 aa, Roseburia sp.
KLCKLVTAY

SEQ ID NO: 35 - protein, 9 aa, Roseburia sp.
FLREHARFY

SEQ ID NO: 36 - protein, 9 aa, Roseburia sp.
LRWLLDGQK

SEQ ID NO: 37 - protein, 9 aa, Roseburia sp.
ARFYIREKL

SEQ ID NO: 38 - protein, 9 aa, Roseburia sp.
YRNYLNPVI

SEQ ID NO: 39 - protein, 9 aa, Roseburia sp.
SEFQAYNPL

SEQ ID NO: 40 - protein, 9 aa, Roseburia sp.
SEQTENPFL

SEQ ID NO: 41 - protein, 9 aa, Roseburia sp.
REKLTELFL

SEQ ID NO: 42 - protein, 9 aa, Roseburia sp.
ESLLVQYQW

SEQ ID NO: 43 - protein, 9 aa, Roseburia sp.
TSDTKQYTY

SEQ ID NO: 44 - protein, 9 aa, Roseburia sp.
GMLNQTTLL

SEQ ID NO: 45 - protein, 9 aa, Roseburia sp.
YIIAVNQTL

SEQ ID NO: 46 - protein, 9 aa, Roseburia sp.
RMSNQQLTV

SEQ ID NO: 47 - protein, 9 aa, Roseburia sp.
AVKAGNMPK

SEQ ID NO: 48 - protein, 9 aa, Roseburia sp.
KTAEEMSQK

SEQ ID NO: 49 - protein, 9 aa, Roseburia sp.
IYQDIDYII

SEQ ID NO: 50 - protein, 9 aa, Roseburia sp.
IIIDYTAAY

SEQ ID NO: 51 - protein, 9 aa, Roseburia sp.
MRVTNNMML

SEQ ID NO: 52 - protein, 9 aa, Roseburia sp.
YRTNCKLTF

SEQ ID NO: 53 - protein, 9 aa, Roseburia sp.
VELKTAEEM

SEQ ID NO: 54 - protein, 9 aa, Roseburia sp.
SAQENLQTW

SEQ ID NO: 55 - protein, 9 aa, Roseburia sp.
KTGTLSYHY

SEQ ID NO: 56 - protein, 9 aa, Roseburia sp.
FSDEGKMSY

SEQ ID NO: 57 - protein, 9 aa, Roseburia sp.
KLCDIYSEL

SEQ ID NO: 58 - protein, 9 aa, Roseburia sp.
VLAKAQFAI

SEQ ID NO: 59 - protein, 9 aa, Roseburia sp.
KLDDRIANA

SEQ ID NO: 60 - protein, 9 aa, Roseburia sp.
ISFDEAFHV

SEQ ID NO: 61 - protein, 9 aa, Roseburia sp.
ILRVPSYYK

SEQ ID NO: 62 - protein, 9 aa, Roseburia sp.
KTFQCIADK

SEQ ID NO: 63 - protein, 9 aa, Roseburia sp.
SYYKTFQCI

SEQ ID NO: 64 - protein, 9 aa, Roseburia sp.
RYFANGKSF

SEQ ID NO: 65 - protein, 9 aa, Roseburia sp.
YYMGIEGAF

SEQ ID NO: 66 - protein, 9 aa, Roseburia sp.
YFHVRMETF

SEQ ID NO: 67 - protein, 9 aa, Roseburia sp.
VYFTYRYFM

SEQ ID NO: 68 - protein, 9 aa, Roseburia sp.
RVPSYYKTF

SEQ ID NO: 69 - protein, 9 aa, Roseburia sp.
DVREKSLSV

SEQ ID NO: 70 - protein, 9 aa, Roseburia sp.
MILRVPSYY

SEQ ID NO: 71 - protein, 9 aa, Roseburia sp.
ALCEVCTEY

SEQ ID NO: 72 - protein, 9 aa, Roseburia sp.
YRYFMRAWY

SEQ ID NO: 73 - protein, 9 aa, Roseburia sp.
YRTQAVAIL

SEQ ID NO: 74 - protein, 9 aa, Roseburia sp.
VRMETFDEL

SEQ ID NO: 75 - protein, 9 aa, Roseburia sp.
NEIWYEHIL

SEQ ID NO: 76 - protein, 9 aa, Roseburia sp.
YEDIELPDL

SEQ ID NO: 77 - protein, 9 aa, Roseburia sp.
IEGAFGERL

SEQ ID NO: 78 - protein, 9 aa, Roseburia sp.
KSGDYNEIW

SEQ ID NO: 79 - protein, 9 aa, Roseburia sp.
RLDSGNYNV

SEQ ID NO: 80 - protein, 9 aa, Roseburia sp.
KLLEKYNAL

SEQ ID NO: 81 - protein, 9 aa, Roseburia sp.
KTRKRISRK

SEQ ID NO: 82 - protein, 9 aa, Roseburia sp.
DAIMRVEAY

SEQ ID NO: 83 - protein, 9 aa, Clostridium sp.
TSENMTSAY

SEQ ID NO: 84 - protein, 9 aa, Clostridium sp.
STDVPVKEY

SEQ ID NO: 85 - protein, 9 aa, Clostridium sp.
AMTEISEML

SEQ ID NO: 86 - protein, 9 aa, Clostridium sp.
KLLNGEYDL

SEQ ID NO: 87 - protein, 9 aa, Clostridium sp.
VLEVNIPAV

SEQ ID NO: 88 - protein, 9 aa, Clostridium sp.
RMNAQIEGL

SEQ ID NO: 89 - protein, 9 aa, Clostridium sp.
TIKSIPLTK

SEQ ID NO: 90 - protein, 9 aa, Clostridium sp.
DMAEEMTSY

SEQ ID NO: 91 - protein, 9 aa, Clostridium sp.
RPSQVLQLL

SEQ ID NO: 92 - protein, 9 aa, Clostridium sp.
EMLQRINEL

SEQ ID NO: 93 - protein, 9 aa, Clostridium sp.
GQKLLNGEY

SEQ ID NO: 94 - protein, 9 aa, Clostridium sp.
MRLDVSGAL

SEQ ID NO: 95 - protein, 9 aa, Clostridium sp.
GENGFEMRL

SEQ ID NO: 96 - protein, 9 aa, Roseburia sp.
RIRDTDMAK

SEQ ID NO: 97 - protein, 9 aa, Roseburia sp.
KVSSQRSAL

SEQ ID NO: 98 - protein, 9 aa, Roseburia sp.
VKSSLAFSL

SEQ ID NO: 99 - protein, 9 aa, Roseburia sp.
LADFIYQKY

SEQ ID NO: 100 - protein, 9 aa, Roseburia sp.
AVAEILAMV

SEQ ID NO: 101 - protein, 9 aa, Roseburia sp.
LMSDALIQI

SEQ ID NO: 102 - protein, 9 aa, Roseburia sp.
FVVTALISV

SEQ ID NO: 103 - protein, 9 aa, Roseburia sp.
RMMQDVPKA

SEQ ID NO: 104 - protein, 9 aa, Roseburia sp.
YLAQKIKEA

SEQ ID NO: 105 - protein, 9 aa, Roseburia sp.
GLADFIYQK

SEQ ID NO: 106 - protein, 9 aa, Roseburia sp.
LYQAVAEIL

SEQ ID NO: 107 - protein, 9 aa, Roseburia sp.
LMNSFVDIY

SEQ ID NO: 108 - protein, 9 aa, Roseburia sp.
KSKELTAAF

SEQ ID NO: 109 - protein, 9 aa, Roseburia sp.
RIFSKDSIF

SEQ ID NO: 110 - protein, 9 aa, Roseburia sp.
QQKQLHLIM

SEQ ID NO: 111 - protein, 9 aa, Roseburia sp.
RRMMQDVPK

SEQ ID NO: 112 - protein, 9 aa, Roseburia sp.
GHAQDIFIL

SEQ ID NO: 113 - protein, 9 aa, Roseburia sp.
YEIPLMQAI

SEQ ID NO: 114 - protein, 9 aa, Roseburia sp.
KELTAAFDL

SEQ ID NO: 115 - protein, 9 aa, Roseburia sp.
IEIVENKPL

SEQ ID NO: 116 - protein, 9 aa, Roseburia sp.
GEDYLAQKI

SEQ ID NO: 117 - protein, 9 aa, Roseburia sp.
LIMEWDLQW

SEQ ID NO: 118 - protein, 9 aa, Roseburia sp.
LISVIQVGW

SEQ ID NO: 119 - protein, 9 aa, Roseburia sp.
KQLHLIMEW

SEQ ID NO: 120 - protein, 9 aa, Roseburia sp.
FTGLQASRY

SEQ ID NO: 121 - protein, 9 aa, Roseburia sp.
ALDDAIAMV

SEQ ID NO: 122 - protein, 9 aa, Roseburia sp.
SIFSSTATV

SEQ ID NO: 123 - protein, 9 aa, Roseburia sp.
KMQAQIDAL

SEQ ID NO: 124 - protein, 9 aa, Roseburia sp.
SLVLTFSGK

SEQ ID NO: 125 - protein, 9 aa, Roseburia sp.
NMSAVITNK

SEQ ID NO: 126 - protein, 9 aa, Roseburia sp.
TIKQPAATK

SEQ ID NO: 127 - protein, 9 aa, Roseburia sp.
ETSAILQRM

SEQ ID NO: 128 - protein, 9 aa, Roseburia sp.
DMAEEMTNY

SEQ ID NO: 129 - protein, 9 aa, Roseburia sp.
LPQNVLSLL

SEQ ID NO: 130 - protein, 9 aa, Roseburia sp.
LQRMRELSV

SEQ ID NO: 131 - protein, 9 aa, Roseburia sp.
LQQAGVSVL

SEQ ID NO: 132 - protein, 9 aa, Roseburia sp.
SRYGSSASL

SEQ ID NO: 133 - protein, 9 aa, Roseburia sp.
VELSAGTAI

SEQ ID NO: 134 - protein, 9 aa, Roseburia sp.
TEYNSKSLL

SEQ ID NO: 135 - protein, 9 aa, Roseburia sp.
SSASLVLTF

SEQ ID NO: 136 - protein, 9 aa, unidentified
TSENMTAAY

SEQ ID NO: 137 - protein, 9 aa, unidentified
KLLNGEFDL

SEQ ID NO: 138 - protein, 9 aa, unidentified
GQKLLNGEF

SEQ ID NO: 139 - protein, 9 aa, unidentified
MRLDVSEAK

SEQ ID NO: 140 - protein, 9 aa, Clostridium sp.
ILVMVTVTV

SEQ ID NO: 141 - protein, 9 aa, Clostridium sp.
LQGPFVINV

SEQ ID NO: 142 - protein, 9 aa, Clostridium sp.
MTVNLQGPF

SEQ ID NO: 143 - protein, 9 aa, Roseburia sp.
LTRKKGEAL